European Patent Specification EP 3 368 553 B1, published August 2, 2023. Title: POLYMER-BASED THERAPEUTICS FOR INDUCTIVE BROWNING OF FAT. Applicant: Purdue  Research Foundation. The sequence listing filed with the application follows.

SEQUENCE LISTING (20 sequences)

SEQ ID NO: 1 - DNA, 24 bp, artificial
  Hey1 forward
tgaatccagatgaccagctactgt

SEQ ID NO: 2 - DNA, 24 bp, artificial
  Hey1 reverse
tactttcagactccgatcgcttac

SEQ ID NO: 3 - DNA, 20 bp, artificial
  HeyL forward
cagatgcaagcccggaagaa

SEQ ID NO: 4 - DNA, 20 bp, artificial
  HeyL reverse
accagaggcatggagcatct

SEQ ID NO: 5 - DNA, 21 bp, artificial
  Hes1 forward
gcacagaaagtcatcaaagcc

SEQ ID NO: 6 - DNA, 21 bp, artificial
  Hes1 reverse
ttgatctgggtcatgcagttg

SEQ ID NO: 7 - DNA, 21 bp, artificial
  UCP1 forward
aggcttccagtaccattaggt

SEQ ID NO: 8 - DNA, 22 bp, artificial
  UCP1 reverse
ctgagtgaggcaaagctgattt

SEQ ID NO: 9 - DNA, 22 bp, artificial
  Ppargc1a forward
agccgtgaccactgacaacgag

SEQ ID NO: 10 - DNA, 23 bp, artificial
  Ppargc1a reverse
gctgcatggttctgagtgctaag

SEQ ID NO: 11 - DNA, 22 bp, artificial
  Cidea forward
tgacattcatgggattgcagac

SEQ ID NO: 12 - DNA, 22 bp, artificial
  Cidea reverse
ggccagttgtgatgactaagac

SEQ ID NO: 13 - DNA, 22 bp, artificial
  Dio2 forward
aattatgcctcggagaagaccg

SEQ ID NO: 14 - DNA, 21 bp, artificial
  Dio2 reverse
ggcagttgcctagtgaaaggt

SEQ ID NO: 15 - DNA, 21 bp, artificial
  Cox5b forward
ttcaaggttacttcgcggagt

SEQ ID NO: 16 - DNA, 22 bp, artificial
  Cos5b reverse
cgggactagattagggtcttcc

SEQ ID NO: 17 - DNA, 21 bp, artificial
  Cox7a forward
gctctggtccggtcttttagc

SEQ ID NO: 18 - DNA, 21 bp, artificial
  Cox7a reverse
gtactgggaggtcattgtcgg

SEQ ID NO: 19 - protein, 5 aa, artificial
  tumor targeting peptide
CGKRK

SEQ ID NO: 20 - protein, 9 aa, artificial
  peptide interacting with prohibitin
CKGGRAKDC